European Patent Application EP 4 248 757 A2, published September 27, 2023. Title: IMPROVED ENZYMATIC MODIFICATION OF PHOSPHOLIPIDS IN FOOD. Applicant: DuPont Nutrition Biosciences ApS. The sequence listing filed with the application follows.

SEQUENCE LISTING (26 sequences)

SEQ ID NO: 1 - protein, 186 aa, Trichoderma harzianum
MKFAALLATLAPAVLALPASDAALTRRQTSLSTITDQYLFSLTLPDFISRRNAKNPATLDWTSDGCTSSPDNPFGFPFVPACYRHDFGYQNYRIQNRFTESGKLSIDNNFKADLYFQCQTSSVQSVCNALADVYYAAVRAFGGGDASPGKREQSQEDLVKVYEEKLEIYNNAVKDAQDKGLLPILE

SEQ ID NO: 2 - protein, 170 aa, Trichoderma harzianum
LPASDAALTRRQTSLSTITDQYLFSLTLPDFISRRNAKNPATLDWTSDGCTSSPDNPFGFPFVPACYRHDFGYQNYRIQNRFTESGKLSIDNNFKADLYFQCQTSSVQSVCNALADVYYAAVRAFGGGDASPGKREQSQEDLVKVYEEKLEIYNNAVKDAQDKGLLPILE

SEQ ID NO: 3 - protein, 180 aa, Pestalotiopsis fici
MRFISTLSLCILPAAALAVPVADKRQDDVEAVTDEILFDITLPEFTTRRNAEDPSYLDWTSDGCTDSPDNPLGFPYEPACNRHDFGYTNYREQSRFTVSAKASIDSNFKDDLYYQCEVNGSFESICEALADVYYAAVVEFGGDDATPGKRSSLYEEKLAIYNQLVAEAVAKGELVLPETA

SEQ ID NO: 4 - protein, 162 aa, Pestalotiopsis fici
VPVADKRQDDVEAVTDEILFDITLPEFTTRRNAEDPSYLDWTSDGCTDSPDNPLGFPYEPACNRHDFGYTNYREQSRFTVSAKASIDSNFKDDLYYQCEVNGSFESICEALADVYYAAVVEFGGDDATPGKRSSLYEEKLAIYNQLVAEAVAKGELVLPETA

SEQ ID NO: 5 - protein, 177 aa, Metarhizium guizhouense
MKLNTTLLALATTALAAPASDVTTPKRQDINTVTDQLLFSSTLSQFEARRNAKEPPSLDWSSDGCTSSPDNPFGFPFLPACHRHDFGYQNYRIQKRFTKAAKAKIDSNFKTDLYYQCRSVSAKDACNGLADVYYEAVKEFGGGDATKRDRSDYDRAVAAYNAAVKEAQEQGLLPILD

SEQ ID NO: 6 - protein, 161 aa, Metarhizium guizhouense
APASDVTTPKRQDINTVTDQLLFSSTLSQFEARRNAKEPPSLDWSSDGCTSSPDNPFGFPFLPACHRHDFGYQNYRIQKRFTKAAKAKIDSNFKTDLYYQCRSVSAKDACNGLADVYYEAVKEFGGGDATKRDRSDYDRAVAAYNAAVKEAQEQGLLPILD

SEQ ID NO: 7 - protein, 184 aa, Diaporthe ampelina
MKVSSIACVAWLVPATFALGPVPLSPRQDIQTVTDSYLFDISLAQFITYRDAQNPSTLDWTSDGCSDSPDNPLGFNFEPACYRHDFGYTNYRAQSRFTKAAKASIDTNFQEDLKFQCESESFESICDALADVYYTAVKLFGGQDATKRADSEDVDADALAEYEHAVAVYEQLVAEAKANGEIPA

SEQ ID NO: 8 - protein, 166 aa, Diaporthe ampelina
LGPVPLSPRQDIQTVTDSYLFDISLAQFITYRDAQNPSTLDWTSDGCSDSPDNPLGFNFEPACYRHDFGYTNYRAQSRFTKAAKASIDTNFQEDLKFQCESESFESICDALADVYYTAVKLFGGQDATKRADSEDVDADALAEYEHAVAVYEQLVAEAKANGEIPA

SEQ ID NO: 9 - protein, 187 aa, Magnaporthe oryzae
MAGDNVGFGLMKFLALLAAAVTVLASPLQMERRQSDLVAITDKLLYSTSLPDFVARRNARDPPSLDWTSDGCTSSPDNPLGFPFTPACNRHDFGYQNYRIQSRFTQSNKFNIDNNFLLDLNNQCNGLNIIARGTCRALADVYYAAVRAFGGSDATPGKRNEDLEKEYNEKLAIYNVLLAEAKKGNYI

SEQ ID NO: 10 - protein, 162 aa, Magnaporthe oryzae
SPLQMERRQSDLVAITDKLLYSTSLPDFVARRNARDPPSLDWTSDGCTSSPDNPLGFPFTPACNRHDFGYQNYRIQSRFTQSNKFNIDNNFLLDLNNQCNGLNIIARGTCRALADVYYAAVRAFGGSDATPGKRNEDLEKEYNEKLAIYNVLLAEAKKGNYI

SEQ ID NO: 11 - protein, 184 aa, Neonectria ditissima
MKFTAPFLVFLSGAAAFPAREIASSVVGRATIQETTDELLFSVTLPQFTVRRNALNPPTLDWTSDGCTSSPDNPFGFPFVPACNRHDFGYNNYRIQTRFTVSAKAKIDSNFKTDLYYQCSSVSATSVCNALADVYYAAVRAFGGDDATPGKRTEDLVKIYEEKVAIYNSLVEEAQKNGELPILE

SEQ ID NO: 12 - protein, 168 aa, Neonectria ditissima
FPAREIASSVVGRATIQETTDELLFSVTLPQFTVRRNALNPPTLDWTSDGCTSSPDNPFGFPFVPACNRHDFGYNNYRIQTRFTVSAKAKIDSNFKTDLYYQCSSVSATSVCNALADVYYAAVRAFGGDDATPGKRTEDLVKIYEEKVAIYNSLVEEAQKNGELPILE

SEQ ID NO: 13 - protein, 187 aa, Trichoderma gamsii
MKLATLFFTLAPAALALPASKESPTRRQSDLVAITDQLLFNTTLPDFITHRNAQDPSTLDWTSDGCTDSPDNPFGFPYVPACNRHDFGYQNYRLQNRFTDSGKLNIDNNFKSDLYYQCQSVSAQSACEDLADVYYAAVRAFGGGDSSPGRRDESHEDLVKEYEAKLEIYHQAVKEAQEKGLLPILDQ

SEQ ID NO: 14 - protein, 171 aa, Trichoderma gamsii
LPASKESPTRRQSDLVAITDQLLFNTTLPDFITHRNAQDPSTLDWTSDGCTDSPDNPFGFPYVPACNRHDFGYQNYRLQNRFTDSGKLNIDNNFKSDLYYQCQSVSAQSACEDLADVYYAAVRAFGGGDSSPGRRDESHEDLVKEYEAKLEIYHQAVKEAQEKGLLPILDQ

SEQ ID NO: 15 - protein, 178 aa, Metarhizium anisopliae
MKFNNAILLALATTVLAAPASDVTTPKRQDINTVTDQLLFSSSLPQFEARRNANDPPLLDWSSDGCTSSPDNPFGFPFLPACHRHDFGYQNYRIQTRFTKAAKAKIDSNFKSDLYYQCQSVSAKNACDRLADVYYEAVKEFGGGDATKRDRSDFDRAVAAYNAAVKEAQEQGLLPVLD

SEQ ID NO: 16 - protein, 161 aa, Metarhizium anisopliae
APASDVTTPKRQDINTVTDQLLFSSSLPQFEARRNANDPPLLDWSSDGCTSSPDNPFGFPFLPACHRHDFGYQNYRIQTRFTKAAKAKIDSNFKSDLYYQCQSVSAKNACDRLADVYYEAVKEFGGGDATKRDRSDFDRAVAAYNAAVKEAQEQGLLPVLD

SEQ ID NO: 17 - protein, 279 aa, Fusarium heterosporum
EAEAAVGVTSTDFTNFKFYIQHGAAAYCNSGTAAGAKITCSNNGCPTIESNGVTVVASFTGSKTGIGGYVSTDSSRKEIVVAIRGSSNIRNWLTNLDFDQSDCSLVSGCGVHSGFQNAWAEISAQASAAVAKARKANPSFKVVATGHSLGGAVATLSAANLRAAGTPVDIYTYGAPRVGNAALSAFISNQAGGEFRVTHDKDPVPRLPPLIFGYRHTTPEYWLSGGGGDKVDYAISDVKVCEGAANLMCNGGTLGLDIDAHLHYFQATDACNAGGFSWR

SEQ ID NO: 18 - protein, 346 aa, Fusarium oxysporum
MLLLPLLSAITLAVASPVALDDYVNSLEERAVGVTTTDFSNFKFYIQHGAAAYCNSEAAAGSKITCSNNGCPTVQGNGATIVTSFVGSKTGIGGYVATDSARKEIVVSFRGSINIRNWLTNLDFGQEDCSLVSGCGVHSGFQRAWNEISSQATAAVASARKANPSFNVISTGHSLGGAVAVLAAANLRVGGTPVDIYTYGSPRVGNAQLSAFVSNQAGGEYRVTHADDPVPRLPPLIFGYRHTTPEFWLSGGGGDKVDYTISDVKVCEGAANLGCNGGTLGLDIAAHLHYFQATDACNAGGFSWRRYRSAESVDKRATMTDAELEKKLNSYVQMDKEYVKNNQARS

SEQ ID NO: 19 - DNA, 558 bp, Trichoderma harzianum
  source 1..558: mol_type = unassigned DNA
atgaagttcgccgccctgctggccaccctggcccccgccgtcctggccctccccgcctctgacgccgccctcacccgacgacagacctctctgagcaccatcaccgaccagtacctgttcagcctcaccctccctgacttcatctctcgacgaaacgccaagaaccctgccaccctggactggacctctgacggctgcaccagctctcctgacaaccctttcggcttccctttcgtccccgcctgctaccgacacgacttcggctaccagaactaccgcatccagaaccgattcaccgagtccggcaagctcagcatcgacaacaacttcaaggccgacctgtacttccagtgccagaccagctccgtccagtctgtctgcaacgccctggccgacgtctactacgccgccgtccgagccttcggcggcggcgacgccagccccggcaagcgcgagcagtctcaggaggacctcgtcaaggtctacgaggagaagctggagatctacaacaacgccgtcaaggacgcccaggacaagggcctgctgcctatcctcgag

SEQ ID NO: 20 - DNA, 540 bp, Pestalotiopsis fici
  source 1..540: mol_type = unassigned DNA
atgcgcttcatcagcaccctgtctctgtgcatcctccccgccgccgccctcgccgtccccgtcgccgacaagcgccaggacgacgtcgaggccgtcaccgacgagatcctgttcgacatcaccctgcctgagttcaccacccgacgcaacgccgaggacccttcttacctggactggacctctgacggctgcaccgactctcctgacaaccctctgggcttcccttacgagcctgcctgcaaccgacacgacttcggctacaccaactaccgcgagcagtctcgattcaccgtctctgccaaggccagcatcgactctaacttcaaggacgacctgtactaccagtgcgaggtcaacggctctttcgagtctatctgcgaggccctcgccgacgtctactacgccgccgtcgtcgagttcggcggcgacgacgccacccccggcaagcgatctagcctgtacgaagaaaagctggccatctacaaccagctggtcgccgaggccgtcgccaagggcgagctggtcctccctgagaccgcc

SEQ ID NO: 21 - DNA, 531 bp, Metarhizium guizhouense
  source 1..531: mol_type = unassigned DNA
atgaagctcaacaccaccctcctggccctggccaccaccgccctcgccgcccctgcctctgacgtcaccacccctaagcgacaggacatcaacaccgtcaccgaccagctgctgttcagctctaccctgtctcagttcgaggcccgacgaaacgccaaagagcctccttctctggactggtcttctgacggctgcacctctagccctgacaaccctttcggcttccctttcctccccgcctgccaccgacacgacttcggctaccagaactaccgcatccagaagcgattcaccaaggccgccaaggccaagatcgactctaacttcaagaccgacctgtactaccagtgccgcagcgtctctgccaaggacgcctgcaacggcctcgccgacgtctactacgaggccgtcaaggaatttggcggcggcgacgccaccaagcgagaccgatctgactacgaccgagccgtcgccgcctacaacgccgccgtcaaagaggcccaggaacagggcctgctccccatcctggac

SEQ ID NO: 22 - DNA, 552 bp, Diaporthe ampelina
  source 1..552: mol_type = unassigned DNA
atgaaggtctcctctattgcctgcgttgcttggctcgtccccgctaccttcgccctgggccccgtccctctgtctcctcgccaggacattcagaccgttaccgactcttacctgttcgacattagcctggctcagttcatcacctaccgagacgcccagaaccctagcaccctggactggacctccgacggctgcagcgacagccccgacaaccctctgggcttcaacttcgagcctgcttgctaccgccacgacttcggctacaccaactaccgcgctcagtctcgattcaccaaggccgctaaggcttctattgacaccaacttccaggaagacctcaagttccagtgcgagtctgagtctttcgagtccatttgcgacgctctcgccgacgtctactacaccgccgttaagctgttcggcggccaggacgccaccaaacgagctgactccgaggacgttgacgctgacgctctcgctgagtacgagcacgctgttgccgtttacgagcagctcgttgctgaggccaaggctaacggcgagatccctgcc

SEQ ID NO: 23 - DNA, 561 bp, Magnaporthe oryzae
  source 1..561: mol_type = unassigned DNA
atggcgggtgacaacgtcggcttcggcctgatgaagttcctcgctctcctcgccgctgctgttaccgttctggcttctcctctgcagatggagcgccgacagtctgacctcgtcgccattaccgacaagctgctgtactctaccagcctccccgacttcgttgctcgccgaaacgctcgtgaccctcctagcctggactggaccagcgacggctgcacctctagccctgacaaccctctgggcttccctttcacccccgcttgcaaccgccacgacttcggctaccagaactaccgcatccagtctcgattcacccagtctaacaagttcaacattgacaacaacttcctgctcgacctgaacaaccagtgcaacggcctgaacatcattgcccgaggcacctgccgcgctctggctgacgtttactacgctgccgtccgcgctttcggcggcagcgacgccacccccggcaagcgaaacgaggacctggagaaagagtacaacgagaagctcgctatatataacgttctcctggctgaggccaagaagggcaactacatc

SEQ ID NO: 24 - DNA, 552 bp, Neonectria ditissima
  source 1..552: mol_type = unassigned DNA
atgaagttcactgctcctttcctggttttcctcagcggcgccgctgccttccccgctcgcgagattgcatctagcgtcgttggccgcgctaccatccaagagaccactgacgagctcctgttctctgttactctgcctcagttcaccgtccgccgaaacgctcttaaccctcccactcttgactggacttctgacggctgcactagcagccctgacaaccctttcggcttccctttcgtccccgcttgcaaccgacacgacttcggctacaacaactaccgcatccagactcgattcaccgttagcgctaaggccaagatcgactctaacttcaagaccgacctgtactaccagtgctctagcgtctctgccacctccgtttgcaacgccctggctgacgtttactacgctgctgtccgagctttcggcggcgacgacgccacccccggcaagcgaactgaggacctggttaagatctacgaagagaaggtcgccatctacaacagccttgttgaggaagcccagaagaacggcgagcttcctattcttgag

SEQ ID NO: 25 - DNA, 561 bp, Trichoderma gamsii
  source 1..561: mol_type = unassigned DNA
atgaagctggctaccctgttcttcaccctcgcccctgctgctctggctctccccgcttctaaagaatctcctacccgccgacagtctgacctcgttgctatcaccgaccagctcctgttcaacaccaccctgcctgacttcattacccaccgaaacgctcaggaccctagcaccctcgactggacctctgacggctgcaccgactctcctgacaaccctttcggcttcccttacgtccccgcttgcaaccgccacgacttcggctaccagaactaccgactgcagaaccgattcaccgacagcggcaagctgaacattgacaacaacttcaagagcgacctgtactaccagtgccagtccgttagcgcccagagcgcttgcgaggacctcgctgacgtttactacgccgctgttcgcgctttcggcggcggcgacagcagccccggccgccgagacgagtctcacgaggacctcgttaaggaatacgaggccaagctggagatctaccaccaggccgtcaaagaagctcaagaaaagggcctcctgcctattctggaccag

SEQ ID NO: 26 - DNA, 534 bp, Metarhizium anisopliae
  source 1..534: mol_type = unassigned DNA
atgaagttcaacaacgccatcctcctggctctcgccaccaccgttctcgccgcccccgcttctgacgtcaccacccctaagcgacaggacattaacaccgttaccgaccagctcctgttctctagcagcctccctcagttcgaggctcgccgaaacgctaacgaccctcctctgctggactggtctagcgacggctgcacctctagccctgacaaccctttcggcttccctttcctgcctgcttgccaccgacacgacttcggctaccagaactaccgcattcagacccgattcaccaaggccgctaaggctaagattgacagcaacttcaagtctgacctgtactaccagtgccagagcgtttccgccaagaacgcttgcgaccgactcgctgacgtttactacgaggccgtcaaagaatttggcggcggcgacgctaccaagcgagaccgatctgacttcgaccgcgctgttgctgcttacaacgctgccgttaaggaagcccaagagcagggcctgctccccgtcctggac